European Patent Specification EP 3 737 702 B1, published July 29, 2026. Title: SUBCUTANEOUS DOSING OF ANTI-CD38 ANTIBODIES. Applicant: Takeda Pharmaceutical Company Limited Dahl, Martin Fedyk, Eric Evans, Robert Zhao, Lin. Application Filed herewith. The sequence listing filed with the application follows.

SEQUENCE LISTING (13 sequences)

SEQ ID NO: 1 - protein, 300 aa, Artificial Sequence
  Human CD38
MANCEFSPVSGDKPCCRLSRRAQLCLGVSILVLILVVVLAVVVPRWRQQWSGPGTTKRFPETVLARCVKYTEIHPEMRHVDCQSVWDAFKGAFISKHPCNITEEDYQPLMKLGTQTVPCNKILLWSRIKDLAHQFTQVQRDMFTLEDTLLGYLADDLTWCGEFNTSKINYQSCPDWRKDCSNNPVSVFWKTVSRRFAEAACDVVHVMLNGSRSKIFDKNSTFGSVEVHNLQPEKVQTLEAWVIHGGREDSRDLCQDPTIKELESIISKRNIQFSCKNIYRPDKFLQCVKNPEDSSCTSEI

SEQ ID NO: 2 - protein, 301 aa, Artificial Sequence
  Cyno CD38
MANCEFSPVSGDKPCCRLSRRAQVCLGVCLLVLLILVVVVAVVLPRWRQQWSGSGTTSRFPETVLARCVKYTEVHPEMRHVDCQSVWDAFKGAFISKYPCNITEEDYQPLVKLGTQTVPCNKTLLWSRIKDLAHQFTQVQRDMFTLEDMLLGYLADDLTWCGEFNTFEINYQSCPDWRKDCSNNPVSVFWKTVSRRFAETACGVVHVMLNGSRSKIFDKNSTFGSVEVHNLQPEKVQALEAWVIHGGREDSRDLCQDPTIKELESIISKRNIRFFCKNIYRPDKFLQCVKNPEDSSCLSGI

SEQ ID NO: 3 - protein, 8 aa, Artificial Sequence
  HCDR1 AB79
GFTFDDYG

SEQ ID NO: 4 - protein, 8 aa, Artificial Sequence
  HCDR2 AB79
ISWNGGKT

SEQ ID NO: 5 - protein, 16 aa, Artificial Sequence
  HCDR3 AB79
ARGSLFHDSSGFYFGH

SEQ ID NO: 6 - protein, 8 aa, Artificial Sequence
  LCDR1 AB79
SSNIGDNY

SEQ ID NO: 7 - protein, 3 aa, Artificial Sequence
  LCDR2 AB79
RDS

SEQ ID NO: 8 - protein, 10 aa, Artificial Sequence
  LCDR3 AB79
QSYDSSLSGS

SEQ ID NO: 9 - protein, 135 aa, Artificial Sequence
  (VH) chain amino acid sequence
EVQLLESGGGLVQPGGSLRLSCAASGFTFDDYGMSWVRQAPGKGLEWVSDISWNGGKTHYVDSVKGQFTISRDNSKNTLYLQMNSLRAEDTAVYYCARGSLFHDSSGFYFGHWGQGTLVTVSSASTKGPSVFPLA

SEQ ID NO: 10 - protein, 129 aa, Artificial Sequence
  (VL) chain amino acid sequence
QSVLTQPPSASGTPGQRVTISCSGSSSNIGDNYVSWYQQLPGTAPKLLIYRDSQRPSGVPDRFSGSKSGTSASLAISGLRSEDEADYYCQSYDSSLSGSVFGGGTKLTVLGQPKANPTVTLFPPSSEEL

SEQ ID NO: 11 - protein, 453 aa, Artificial Sequence
  (HC) amino acid sequence
EVQLLESGGGLVQPGGSLRLSCAASGFTFDDYGMSWVRQAPGKGLEWVSDISWNGGKTHYVDSVKGQFTISRDNSKNTLYLQMNSLRAEDTAVYYCARGSLFHDSSGFYFGHWGQGTLVTVSSASTKGPSVFPLAPSSKSTSGGTAALGCLVKDYFPEPVTVSWNSGALTSGVHTFPAVLQSSGLYSLSSVVTVPSSSLGTQTYICNVNHKPSNTKVDKRVEPKSCDKTHTCPPCPAPELLGGPSVFLFPPKPKDTLMISRTPEVTCVVVDVSHEDPEVKFNWYVDGVEVHNAKTKPREEQYNSTYRVVSVLTVLHQDWLNGKEYKCKVSNKALPAPIEKTISKAKGQPREPQVYTLPPSREEMTKNQVSLTCLVKGFYPSDIAVEWESNGQPENNYKTTPPVLDSDGSFFLYSKLTVDKSRWQQGNVFSCSVMHEALHNHYTQKSLSLSPGK

SEQ ID NO: 12 - protein, 216 aa, Artificial Sequence
  (LC) amino acid sequence
QSVLTQPPSASGTPGQRVTISCSGSSSNIGDNYVSWYQQLPGTAPKLLIYRDSQRPSGVPDRFSGSKSGTSASLAISGLRSEDEADYYCQSYDSSLSGSVFGGGTKLTVLGQPKANPTVTLFPPSSEELQANKATLVCLISDFYPGAVTVAWKADGSPVKAGVETTKPSKQSNNKYAASSYLSLTPEQWKSHRSYSCQVTHEGSTVEKTVAPTECS

SEQ ID NO: 13 - protein, 318 aa, Artificial Sequence
  Human CD157
MAAQGCAASRLLQLLLQLLLLLLLLAAGGARARWRGEGTSAHLRDIFLGRCAEYRALLSPEQRNKNCTAIWEAFKVALDKDPCSVLPSDYDLFINLSRHSIPRDKSLFWENSHLLVNSFADNTRRFMPLSDVLYGRVADFLSWCRQKNDSGLDYQSCPTSEDCENNPVDSFWKRASIQYSKDSSGVIHVMLNGSEPTGAYPIKGFFADYEIPNLQKEKITRIEIWVMHEIGGPNVESCGEGSMKVLEKRLKDMGFQYSCINDYRPVKLLQCVDHSTHPDCALKSAAAATQRKAPSLYTEQRAGLIIPLFLVLASRTQL